European Patent Application EP 4 130 044 A1, published February 8, 2023. Title: ANTI-PD1 ANTIBODIES AND THEIR USE AS THERAPEUTICS AND DIAGNOSIS. Applicant: BeiGene Li, Kang Zhang, Tong Song, Jing Xu, Lanlan Liu, Qi Peng, Hao. Application EP. The sequence listing filed with the application follows.

SEQUENCE LISTING (90 sequences)

SEQ ID NO: 1 - DNA, 444 bp, Homo sapiens
ccaggatggttcttagactccccagacaggccctggaacccccccaccttctccccagccctgctcgtggtgaccgaaggggacaacgccaccttcacctgcagcttctccaacacatcggagagcttcgtgctaaactggtaccgcatgagccccagcaaccagacggacaagctggccgccttccccgaggaccgcagccagcccggccaggactgccgcttccgtgtcacacaactgcccaacgggcgtgacttccacatgagcgtggtcagggcccggcgcaatgacagcggcacctacctctgtggggccatctccctggcccccaaggcgcagatcaaagagagcctgcgggcagagctcagggtgacagagagaagggcagaagtgcccacagcccaccccagcccctcacccaggccagccggccagttccaaacc

SEQ ID NO: 2 - protein, 148 aa, Homo sapiens
PGWFLDSPDRPWNPPTFSPALLVVTEGDNATFTCSFSNTSESFVLNWYRMSPSNQTDKLAAFPEDRSQPGQDCRFRVTQLPNGRDFHMSVVRARRNDSGTYLCGAISLAPKAQIKESLRAELRVTERRAEVPTAHPSPSPRPAGQFQT

SEQ ID NO: 3 - DNA, 354 bp, Mus musculus
caggtgcagctgaaggagtcaggacctggcctggtggcgccctcaaagaacctgtccatcacttgcactgtctctgggttttcattaaccagctatggtgtacactggattcgccagcctccaggaaagggactggaatggctgggagtaatatgggccggtggaagcacaaattataattcggctctcatgtccagactgagcatcagcaaagacaactccaggagccaagttttcttaagaatgaacagtctgcaaactgatgacacagccatgtactactgtgccagagcctatggtaactactggtacatcgatgtctggggcgcagggaccacggtcaccgtctcctca

SEQ ID NO: 4 - protein, 118 aa, Mus musculus
QVQLKESGPGLVAPSKNLSITCTVSGFSLTSYGVHWIRQPPGKGLEWLGVIWAGGSTNYNSALMSRLSISKDNSRSQVFLRMNSLQTDDTAMYYCARAYGNYWYIDVWGAGTTVTVSS

SEQ ID NO: 5 - DNA, 321 bp, Mus musculus
gacattgtgatgacccagactcccaaattcctgcttgtatcagcaggagacagggttaccataacctgcaaggccagtcagagtgtgagtaatgatgtagcttggtaccaacagaagccagggcagtctcctaaactgctgataaactatgcatttcatcgcttcactggagtccctgatcgtttcactggcagtggatatgggacggatttcattttcaccatcagcactgtgcaggctgaagacctggcagtttatttctgtcaccaggcttatagttctccgtacacgttcggaggggggaccaagctggaaatgaaa

SEQ ID NO: 6 - protein, 107 aa, Mus musculus
DIVMTQTPKFLLVSAGDRVTITCKASQSVSNDVAWYQQKPGQSPKLLINYAFHRFTGVPDRFTGSGYGTDFIFTISTVQAEDLAVYFCHQAYSSPYTFGGGTKLEMK

SEQ ID NO: 7 - DNA, 342 bp, Mus musculus
cagatccagttggtgcagtctggacctgagctgaagaagcctggagagacagtcaagatctcctgcaaggcttctgggtataccttcacaaactatggaatgaactgggtgaagcaggctccaggaaagggtttaaagtggatgggctggataaacaataataatggagagccaacatatgctgaagagttcaagggacggtttgccttctctttggaaacctctgccagcactgcctatttgcagatcaacaacctcaaaaatgaggacacggctacatatttctgtgcaagagatgttatggactattggggtcaaggaacctcagtcaccgtctcctca

SEQ ID NO: 8 - protein, 114 aa, Mus musculus
QIQLVQSGPELKKPGETVKISCKASGYTFTNYGMNWVKQAPGKGLKWMGWINNNNGEPTYAEEFKGRFAFSLETSASTAYLQINNLKNEDTATYFCARDVMDYWGQGTSVTVSS

SEQ ID NO: 9 - DNA, 330 bp, Mus musculus
gacattgtgctgacccaatctccagcttctttggctgtgtctctagggcagagggccaccatatcctgcagagccagtgaaagtgttgataattatggctatagttttatgcactggtaccagcagaaaccaggacagccaccccaactcctcatctatcgtgcatccaacctagaatctgggatccctgccaggttcagtggcagtgggtctaggacaggcttcaccctcaccattaatcctgtggaggctgatgatgttgcaacctattactgtcagcaaagtaaagaatatccgacgttcggtggaggcaccaagctggaagtcaaa

SEQ ID NO: 10 - protein, 110 aa, Mus musculus
DIVLTQSPASLAVSLGQRATISCRASESVDNYGYSFMHWYQQKPGQPPQLLIYRASNLESGIPARFSGSGSRTGFTLTINPVEADDVATYYCQQSKEYPTFGGGTKLEVK

SEQ ID NO: 11 - protein, 10 aa, Mus musculus
GFSLTSYGVH

SEQ ID NO: 12 - protein, 16 aa, Mus musculus
VIWAGGSTNYNSALMS

SEQ ID NO: 13 - protein, 12 aa, Mus musculus
ARAYGNYWYIDV

SEQ ID NO: 14 - protein, 11 aa, Mus musculus
KASQSVSNDVA

SEQ ID NO: 15 - protein, 7 aa, Mus musculus
YAFHRFT

SEQ ID NO: 16 - protein, 9 aa, Mus musculus
HQAYSSPYT

SEQ ID NO: 17 - protein, 10 aa, Mus musculus
GYTFTNYGMN

SEQ ID NO: 18 - protein, 17 aa, Mus musculus
WINNNNGEPTYAEEFKG

SEQ ID NO: 19 - protein, 7 aa, Mus musculus
ARDVMDY

SEQ ID NO: 20 - protein, 15 aa, Mus musculus
RASESVDNYGYSFMH

SEQ ID NO: 21 - protein, 7 aa, Mus musculus
RASNLES

SEQ ID NO: 22 - protein, 8 aa, Mus musculus
QQSKEYPT

SEQ ID NO: 23 - DNA, 354 bp, Artificial Sequence
  317-4B6 cDNA-Vh
caggtgcagctgcaggagtcgggaccaggactggtgaagccttcggagaccctgtccctcacctgcactgtctctgggttttcattaaccagctatggtgtacactggatccggcagcccccagggaagggactggagtggatcggggtcatatacgccgatggaagcacaaattataatccctccctcaagagtcgagtgaccatatcaaaagacacctccaagaaccaggtttccctgaagctgagctctgtgaccgctgcggacacggccgtgtattactgtgcgagagcctatggtaactactggtacatcgatgtctggggccaagggaccacggtcaccgtctcctca

SEQ ID NO: 24 - protein, 118 aa, Artificial Sequence
  317-4B6 pro-Vh
QVQLQESGPGLVKPSETLSLTCTVSGFSLTSYGVHWIRQPPGKGLEWIGVIYADGSTNYNPSLKSRVTISKDTSKNQVSLKLSSVTAADTAVYYCARAYGNYWYIDVWGQGTTVTVSS

SEQ ID NO: 25 - DNA, 321 bp, Artificial Sequence
  317-4B6 cDNA-Vk
gacatcgtgatgacccagtctccagactccctggctgtgtctctgggcgagagggccaccatcaactgcaagtccagcgagagtgtgagtaatgatgtagcttggtaccagcagaaaccaggacagcctcctaagctgctcattaactatgcatttcatcgcttcactggggtccctgaccgattcagtggcagcgggtatgggacagatttcactctcaccatcagcagcctgcaggctgaagatgtggcagtttattactgtcaccaggcttatagttctccgtacacgtttggccaggggaccaagctggagatcaaa

SEQ ID NO: 26 - protein, 107 aa, Artificial Sequence
  317-4B6 pro-Vk
DIVMTQSPDSLAVSLGERATINCKSSESVSNDVAWYQQKPGQPPKLLINYAFHRFTGVPDRFSGSGYGTDFTLTISSLQAEDVAVYYCHQAYSSPYTFGQGTKLEIK

SEQ ID NO: 27 - DNA, 342 bp, Artificial Sequence
  326-4A3 cDNA-Vh
caggtgcagctggtgcagagcggcagcgagctgaagaagcccggcgccagcgtgaaggtgagctgcaaggccagcggctacaccttcaccaactacggcatgaactgggtgagacaggcccccggccagggcctgaagtggatgggctggatcaacaacaacaacgccgagcccacctacgcccaggacttcagaggcagattcgtgttcagcctggacaccagcgccagcaccgcctacctgcagatcagcagcctgaagaccgaggacaccgccgtgtactactgcgccagagacgtgatggactactggggccagggcaccctggtgaccgtgagcagc

SEQ ID NO: 28 - protein, 114 aa, Artificial Sequence
  326-4A3 pro-Vh
QVQLVQSGSELKKPGASVKVSCKASGYTFTNYGMNWVRQAPGQGLKWMGWINNNNAEPTYAQDFRGRFVFSLDTSASTAYLQISSLKTEDTAVYYCARDVMDYWGQGTLVTVSS

SEQ ID NO: 29 - DNA, 330 bp, Artificial Sequence
  326-4A3 cDNA-Vk
gacattgtgctgacccagtctccagcctccttggccgtgtctccaggacagagggccaccatcacctgcagagccagtgaaagtgttgataattatggctatagttttatgcactggtatcagcagaaaccaggacaacctcctaaactcctgatttaccgtgcatccaacctagaatctggggtcccagccaggttcagcggcagtgggtctgggaccgatttcaccctcacaattaatcctgtggaagctgaggatactgcaaattattactgtcagcaaagtaaagaatatccgacgttcggcggagggaccaaggtggagatcaaa

SEQ ID NO: 30 - protein, 110 aa, Artificial Sequence
  326-4A3 pro-Vk
DIVLTQSPASLAVSPGQRATITCRASESVDNYGYSFMHWYQQKPGQPPKLLIYRASNLESGVPARFSGSGSGTDFTLTINPVEAEDTANYYCQQSKEYPTFGGGTKVEIK

SEQ ID NO: 31 - protein, 10 aa, Mus musculus
GFSLTSYGVH

SEQ ID NO: 32 - protein, 16 aa, Artificial Sequence
  317-4B6 H-CDR2 or CDR-H2
VIYADGSTNYNPSLKS

SEQ ID NO: 33 - protein, 12 aa, Mus musculus
ARAYGNYWYIDV

SEQ ID NO: 34 - protein, 11 aa, Artificial Sequence
  317-4B6 L-CDR1 or CDR-L1
KSSESVSNDVA

SEQ ID NO: 35 - protein, 7 aa, Mus musculus
YAFHRFT

SEQ ID NO: 36 - protein, 9 aa, Mus musculus
HQAYSSPYT

SEQ ID NO: 37 - protein, 10 aa, Mus musculus
GYTFTNYGMN

SEQ ID NO: 38 - protein, 17 aa, Artificial Sequence
  326-4A3 H-CDR2 or CDR-H2
WINNNNAEPTYAQDFRG

SEQ ID NO: 39 - protein, 7 aa, Mus musculus
ARDVMDY

SEQ ID NO: 40 - protein, 15 aa, Mus musculus
RASESVDNYGYSFMH

SEQ ID NO: 41 - protein, 7 aa, Mus musculus
RASNLES

SEQ ID NO: 42 - protein, 8 aa, Mus musculus
QQSKEYPT

SEQ ID NO: 43 - protein, 118 aa, Artificial Sequence
  317-4B2 pro-Vh
QVQLQESGPGLVKPSETLSLTCTVSGFSLTSYGVHWIRQPPGKGLEWIGVIYAGGSTNYNPSLKSRVTISKDTSKNQFSLKLSSVTAADTAVYYCARAYGNYWYIDVWGQGTTVTVSS

SEQ ID NO: 44 - protein, 107 aa, Artificial Sequence; identical to SEQ ID NO: 26
  317-4B2 pro-Vk

SEQ ID NO: 45 - protein, 118 aa, Artificial Sequence
  317-4B5 pro-Vh
QVQLQESGPGLVKPSETLSLTCTVSGFSLTSYGVHWIRQPPGKGLEWIGVIYAGGSTNYNPSLKSRVTISKDTSKNQVSLKLSSVTAADTAVYYCARAYGNYWYIDVWGQGTTVTVSS

SEQ ID NO: 46 - protein, 107 aa, Artificial Sequence; identical to SEQ ID NO: 26
  317-4B5 pro-Vk

SEQ ID NO: 47 - DNA, 354 bp, Artificial Sequence
  317-1 cDNA-Vh
caggtgcagctgcaggagtcgggaccaggactggtgaagccttcggagaccctgtccctcacctgcactgtctctgggttttcattaaccagctatggtgtacactggatccggcagcccccagggaagggactggagtggctgggggtcatatgggccggtggaagcacaaattataatccctccctcaagagtcgactgaccatatcaaaagacaactccaagagccaggtttccctgaagatgagctctgtgaccgctgcggacacggccgtgtattactgtgcgagagcctatggtaactactggtacatcgatgtctggggccaagggaccacggtcaccgtctcctca

SEQ ID NO: 48 - protein, 118 aa, Artificial Sequence
  317-1 pro-Vh
QVQLQESGPGLVKPSETLSLTCTVSGFSLTSYGVHWIRQPPGKGLEWLGVIWAGGSTNYNPSLKSRLTISKDNSKSQVSLKMSSVTAADTAVYYCARAYGNYWYIDVWGQGTTVTVSS

SEQ ID NO: 49 - DNA, 321 bp, Artificial Sequence
  317-1 cDNA-Vk
gacatcgtgatgacccagtctccagactccctggctgtgtctctgggcgagagggccaccatcaactgcaaggccagccagagtgtgagtaatgatgtagcttggtaccagcagaaaccaggacagcctcctaagctgctcattaactatgcatttcatcgcttcactggggtccctgaccgattcagtggcagcgggtatgggacagatttcactctcaccatcagcagcctgcaggctgaagatgtggcagtttattactgtcaccaggcttatagttctccgtacacgtttggcggggggaccaagctggagatcaaa

SEQ ID NO: 50 - protein, 107 aa, Artificial Sequence
  317-1 pro-Vk
DIVMTQSPDSLAVSLGERATINCKASQSVSNDVAWYQQKPGQPPKLLINYAFHRFTGVPDRFSGSGYGTDFTLTISSLQAEDVAVYYCHQAYSSPYTFGGGTKLEIK

SEQ ID NO: 51 - protein, 114 aa, Artificial Sequence
  326-3B1 pro-Vh
QVQLVQSGSELKKPGASVKVSCKASGYTFTNYGMNWVRQAPGQGLKWMGWINNNNGEPTYAQDFRGRFVFSLDTSASTAYLQISSLKTEDTAVYYCARDVMDYWGQGTLVTVSS

SEQ ID NO: 52 - protein, 110 aa, Artificial Sequence
  326-3B1 pro-Vk
DIVLTQSPASLAVSPGQRATITCRASESVDNYGYSFMHWYQQKPGQPPKLLIYRASNLESGVPARFSGSGSRTDFTLTINPVEANDTANYYCQQSKEYPTFGGGTKVEIK

SEQ ID NO: 53 - protein, 114 aa, Artificial Sequence
  326-3G1 pro-Vh
QVQLVQSGPELKKPGASVKVSCKASGYTFTNYGMNWVRQAPGQGLKWMGWINNNNGEPTYAQDFRGRFVFSLDTSASTAYLQISSLKTEDTAVYYCARDVMDYWGQGTLVTVSS

SEQ ID NO: 54 - protein, 110 aa, Artificial Sequence; identical to SEQ ID NO: 52
  326-3G1 pro-Vk

SEQ ID NO: 55 - DNA, 342 bp, Artificial Sequence
  326-1 cDNA-Vh
caggtgcagctggtgcagagcggcagcgagctgaagaagcccggcgccagcgtgaaggtgagctgcaaggccagcggctacaccttcaccaactacggcatgaactgggtgagacaggcccccggccagggcctggagtggatgggctggatcaacaacaacaacggcgagcccacctacgcccagggcttcagaggcagattcgtgttcagcctggacaccagcgccagcaccgcctacctgcagatcagcagcctgaagaccgaggacaccgccgtgtacttctgcgccagagacgtgatggactactggggccagggcaccaccgtgaccgtgagcagc

SEQ ID NO: 56 - protein, 114 aa, Artificial Sequence
  326-1 pro-Vh
QVQLVQSGSELKKPGASVKVSCKASGYTFTNYGMNWVRQAPGQGLEWMGWINNNNGEPTYAQGFRGRFVFSLDTSASTAYLQISSLKTEDTAVYFCARDVMDYWGQGTTVTVSS

SEQ ID NO: 57 - DNA, 330 bp, Artificial Sequence
  326-1 cDNA-Vk
gacattgtgctgacccagtctccagcctccttggccgtgtctccaggacagagggccaccatcacctgcagagccagtgaaagtgttgataattatggctatagttttatgcactggtatcagcagaaaccaggacaacctcctaaactcctgatttaccgtgcatccaacctagaatctggggtcccagccaggttcagcggcagtgggtctaggaccgatttcaccctcacaattaatcctgtggaagctaatgatactgcaaattattactgtcagcaaagtaaagaatatccgacgttcggcggagggaccaaggtggagatcaaa

SEQ ID NO: 58 - protein, 110 aa, Artificial Sequence; identical to SEQ ID NO: 52
  326-1 pro-Vk

SEQ ID NO: 59 - protein, 16 aa, Artificial Sequence
  317-1 H-CDR2 or CDR-H2
VIWAGGSTNYNPSLKS

SEQ ID NO: 60 - protein, 16 aa, Artificial Sequence
  317-4B2 H-CDR2 or CDR-H2
VIYAGGSTNYNPSLKS

SEQ ID NO: 61 - protein, 11 aa, Artificial Sequence
  317-4B2 L-CDR1 or CDR-L1
KSSESVSNDVA

SEQ ID NO: 62 - protein, 17 aa, Artificial Sequence
  326-1 H-CDR2 or CDR-H2
WINNNNGEPTYAQGFRG

SEQ ID NO: 63 - protein, 17 aa, Artificial Sequence
  326-3G1 H-CDR2 or CDR-H2
WINNNNGEPTYAQDFRG

SEQ ID NO: 64 - protein, 118 aa, Artificial Sequence
  317-3A1 pro-Vh
QVQLQESGPGLVKPSETLSLTCTVSGFSLTSYGVHWIRQPPGKGLEWIGVIWAGGSTNYNPSLKSRVTISVDTSKNQFSLKLSSVTAADTAVYYCARAYGNYWYIDVWGQGTTVTVSS

SEQ ID NO: 65 - protein, 118 aa, Artificial Sequence
  317-3C1 pro-Vh
QVQLQESGPGLVKPSETLSLTCTVSGFSLTSYGVHWIRQPPGKGLEWLGVIWAGGSTNYNPSLKSRVTISVDTSKNQFSLKLSSVTAADTAVYYCARAYGNYWYIDVWGQGTTVTVSS

SEQ ID NO: 66 - protein, 118 aa, Artificial Sequence
  317-3E1 pro-Vh
QVQLQESGPGLVKPSETLSLTCTVSGFSLTSYGVHWIRQPPGKGLEWIGVIWAGGSTNYNPSLKSRVTISVDTSKSQFSLKLSSVTAADTAVYYCARAYGNYWYIDVWGQGTTVTVSS

SEQ ID NO: 67 - protein, 118 aa, Artificial Sequence
  317-3F1 pro-Vh
QVQLQESGPGLVKPSETLSLTCTVSGFSLTSYGVHWIRQPPGKGLEWIGVIWAGGSTNYNPSLKSRVTISVDTSKNQVSLKLSSVTAADTAVYYCARAYGNYWYIDVWGQGTTVTVSS

SEQ ID NO: 68 - protein, 118 aa, Artificial Sequence
  317-3G1 pro-Vh
QVQLQESGPGLVKPSETLSLTCTVSGFSLTSYGVHWIRQPPGKGLEWIGVIWAGGSTNYNPSLKSRVTISVDTSKSQVSLKLSSVTAADTAVYYCARAYGNYWYIDVWGQGTTVTVSS

SEQ ID NO: 69 - protein, 118 aa, Artificial Sequence
  317-3H1 pro-Vh
QVQLQESGPGLVKPSETLSLTCTVSGFSLTSYGVHWIRQPPGKGLEWIGVIWAGGSTNYNPSLKSRVTISKDTSKSQVSLKLSSVTAADTAVYYCARAYGNYWYIDVWGQGTTVTVSS

SEQ ID NO: 70 - protein, 118 aa, Artificial Sequence
  317-3I1 pro-Vh
QVQLQESGPGLVKPSETLSLTCTVSGFSLTSYGVHWIRQPPGKGLEWIGVIWAGGSTNYNPSLKSRVTISKDTSKNQVSLKLSSVTAADTAVYYCARAYGNYWYIDVWGQGTTVTVSS

SEQ ID NO: 71 - protein, 118 aa, Artificial Sequence
  317-4B1 pro-Vh
QVQLQESGPGLVKPSETLSLTCTVSGFSLTSYGVHWIRQPPGKGLEWIGVIWAGGSTNYNPSLKSRVTISKDTSKNQFSLKLSSVTAADTAVYYCARAYGNYWYIDVWGQGTTVTVSS

SEQ ID NO: 72 - protein, 118 aa, Artificial Sequence
  317-4B3 pro-Vh
QVQLQESGPGLVKPSETLSLTCTVSGFSLTSYGVHWIRQPPGKGLEWIGVINAGGSTNYNPSLKSRVTISKDTSKNQFSLKLSSVTAADTAVYYCARAYGNYWYIDVWGQGTTVTVSS

SEQ ID NO: 73 - protein, 118 aa, Artificial Sequence
  317-4B4 pro-Vh
QVQLQESGPGLVKPSETLSLTCTVSGFSLTSYGVHWIRQPPGKGLEWIGVIWAGGSTNYNPSLKSRVTISKDTSKNQFSLKLSSVTAADTAVYYCARAYGNYPYIDVWGQGTTVTVSS

SEQ ID NO: 74 - protein, 107 aa, Artificial Sequence
  317-4A2 pro-Vk
DIVMTQSPDSLAVSLGERATINCKSSQSVSNDVAWYQQKPGQPPKLLINYAFHRFTGVPDRFSGSGYGTDFTLTISSLQAEDVAVYYCHQAYSSPYTFGQGTKLEIK

SEQ ID NO: 75 - protein, 114 aa, Artificial Sequence
  326-3A1 pro-Vh
QVQLVQSGPELKKPGASVKVSCKASGYTFTNYGMNWVRQAPGQGLEWMGWINNNNGEPTYAQGFRGRFVFSLDTSASTAYLQISSLKTEDTAVYYCARDVMDYWGQGTLVTVSS

SEQ ID NO: 76 - protein, 114 aa, Artificial Sequence
  326-3C1 pro-Vh
QVQLVQSGPELKKPGASVKVSCKASGYTFTNYGMNWVRQAPGQGLKWMGWINNNNGEPTYAQDFRGRFVFSLDTSASTAYLQISSLKTEDTAVYYCARDVMDYWGQGTTVTVSS

SEQ ID NO: 77 - protein, 114 aa, Artificial Sequence
  326-3D1 pro-Vh
QVQLVQSGSELKKPGASVKVSCKASGYTFTNYGMNWVRQAPGQGLEWMGWINNNNGEPTYAQGFRGRFVFSLDTSASTAYLQISSLKTEDTAVYYCARDVMDYWGQGTLVTVSS

SEQ ID NO: 78 - protein, 114 aa, Artificial Sequence
  326-3E1 pro-Vh
QVQLVQSGSELKKPGASVKVSCKASGYTFTNYGMNWVRQAPGQGLKWMGWINNNNGEPTYAQDFRGRFVFSLDTSASTAYLQISSLKTEDTAVYYCARDVMDYWGQGTTVTVSS

SEQ ID NO: 79 - protein, 114 aa, Artificial Sequence
  326-3F1 pro-Vh
QVQLVQSGPELKKPGASVKVSCKASGYTFTNYGMNWVRQAPGQGLEWMGWINNNNGEPTYAQGFRGRFVFSLDTSASTAYLQISSLKTEDTAVYYCARDVMDYWGQGTTVTVSS

SEQ ID NO: 80 - protein, 114 aa, Artificial Sequence
  326-3B N55D pro-Vh
QVQLVQSGSELKKPGASVKVSCKASGYTFTNYGMNWVRQAPGQGLKWMGWINNNDGEPTYAQDFRGRFVFSLDTSASTAYLQISSLKTEDTAVYYCARDVMDYWGQGTLVTVSS

SEQ ID NO: 81 - protein, 110 aa, Artificial Sequence
  326-4A1 pro-Vk
DIVLTQSPASLAVSPGQRATITCRASESVDNYGYSFMHWYQQKPGQPPKLLIYRASNLESGVPARFSGSGSRTDFTLTINPVEAEDTANYYCQQSKEYPTFGGGTKVEIK

SEQ ID NO: 82 - protein, 110 aa, Artificial Sequence
  326-4A2 pro-Vk
DIVLTQSPASLAVSPGQRATITCRASESVDNYGYSFMHWYQQKPGQPPKLLIYRASNLESGVPARFSGSGSGTDFTLTINPVEANDTANYYCQQSKEYPTFGGGTKVEIK

SEQ ID NO: 83 - protein, 327 aa, Artificial Sequence
  huIgG4mt1 pro
ASTKGPSVFPLAPCSRSTSESTAALGCLVKDYFPEPVTVSWNSGALTSGVHTFPAVLQSSGLYSLSSVVTVPSSSLGTKTYTCNVDHKPSNTKVDKRVESKYGPPCPPCPAPEFEGGPSVFLFPPKPKDTLMISRTPEVTCVVVDVSQEDPEVQFNWYVDGVEVHNAKTKPREEQFNSTYRVVSVLTVLHQDWLNGKEYKCKVSNKGLPSSIEKTISKAKGQPREPQVYTLPPSQEEMTKNQVSLTCLVKGFYPSDIAVEWESNGQPENNYKTTPPVLDSDGSFFLYSRLTVDKSRWQEGNVFSCSVMHEALHNHYTQKSLSLSLGK

SEQ ID NO: 84 - protein, 327 aa, Artificial Sequence
  huIgG4mt2 pro
ASTKGPSVFPLAPCSRSTSESTAALGCLVKDYFPEPVTVSWNSGALTSGVHTFPAVLQSSGLYSLSSVVTVPSSSLGTKTYTCNVDHKPSNTKVDKRVESKYGPPCPPCPAPPVAGGPSVFLFPPKPKDTLMISRTPEVTCVVVDVSQEDPEVQFNWYVDGVEVHNAKTKPREEQFNSTYRVVSVLTVLHQDWLNGKEYKCKVSNKGLPSSIEKTISKAKGQPREPQVYTLPPSQEEMTKNQVSLTCLVKGFYPSDIAVEWESNGQPENNYKTTPPVLDSDGSFFLYSRLTVDKSRWQEGNVFSCSVMHEALHNHYTQKSLSLSLGK

SEQ ID NO: 85 - protein, 327 aa, Artificial Sequence
  huIgG4mt6 pro
ASTKGPSVFPLAPCSRSTSESTAALGCLVKDYFPEPVTVSWNSGALTSGVHTFPAVLQSSGLYSLSSVVTVPSSSLGTKTYTCNVDHKPSNTKVDKRVESKYGPPCPPCPAPPVAGGPSVFLFPPKPKDTLMISRTPEVTCVVVAVSQEDPEVQFNWYVDGVEVHNAKTKPREEQFNSTYRVVSVLTVLHQDWLNGKEYKCKVSNKGLPSSIEKTISKAKGQPREPQVYTLPPSQEEMTKNQVSLTCLVKGFYPSDIAVEWESNGQPENNYKTTPPVLDSDGSFFLYSRLTVDKSRWQEGNVFSCSVMHEALHNHYTQKSLSLSLGK

SEQ ID NO: 86 - protein, 327 aa, Artificial Sequence
  huIgG4mt8 pro
ASTKGPSVFPLAPCSRSTSESTAALGCLVKDYFPEPVTVSWNSGALTSGVHTFPAVLQSSGLYSLSSVVTVPSSSLGTKTYTCNVDHKPSNTKVDKRVESKYGPPCPPCPAPPVAGGPSVFLFPPKPKDTLMISRTPEVTCVVVTVSQEDPEVQFNWYVDGVEVHNAKTKPREEQFNSTYRVVSVLTVLHQDWLNGKEYKCKVSNKGLPSSIEKTISKAKGQPREPQVYTLPPSQEEMTKNQVSLTCLVKGFYPSDIAVEWESNGQPENNYKTTPPVLDSDGSFFLYSRLTVDKSRWQEGNVFSCSVMHEALHNHYTQKSLSLSLGK

SEQ ID NO: 87 - protein, 327 aa, Artificial Sequence
  huIgG4mt9 pro
ASTKGPSVFPLAPCSRSTSESTAALGCLVKDYFPEPVTVSWNSGALTSGVHTFPAVLQSSGLYSLSSVVTVPSSSLGTKTYTCNVDHKPSNTKVDKRVESKYGPPCPPCPAPPVAGGPSVFLFPPKPKDTLMISRTPEVTCVVVAVSQEDPEVQFNWYVDGVEVHNAKTKPREEQFNSTYRVVSVLTVLHQDWLNGKEYKCKVSNKGLPSSIEKTISKAKGQPREPQVYTLPPSQEEMTKNQVSLTCLVKGFYPSDIAVEWESNGQPENNYKTTPPVLDSDGSFFLYSKLTVDKSRWQEGNVFSCSVMHEALHNHYTQKSLSLSLGK

SEQ ID NO: 88 - protein, 327 aa, Artificial Sequence
  huIgG4mt10 pro
ASTKGPSVFPLAPCSRSTSESTAALGCLVKDYFPEPVTVSWNSGALTSGVHTFPAVLQSSGLYSLSSVVTVPSSSLGTKTYTCNVDHKPSNTKVDKRVESKYGPPCPPCPAPPVAGGPSVFLFPPKPKDTLMISRTPEVTCVVVAVSQEDPEVQFNWYVDGVEVHNAKTKPREEQFNSTYRVVSVLTVVHQDWLNGKEYKCKVSNKGLPSSIEKTISKAKGQPREPQVYTLPPSQEEMTKNQVSLTCLVKGFYPSDIAVEWESNGQPENNYKTTPPVLDSDGSFFLYSKLTVDKSRWQEGNVFSCSVMHEALHNHYTQKSLSLSLGK

SEQ ID NO: 89 - protein, 367 aa, Artificial Sequence
  OS8 pro
MERHWIFLLLLSVTAGVHSQVQLQQSGAELARPGASVKMSCKASGYTFTRYTMHWVKQRPGQGLEWIGYINPSRGYTNYNQKFKDKATLTTDKSSSTAYMQLSSLTSEDSAVYYCARYYDDHYCLDYWGQGTTLTVSSGGGGSGGGGSGGGGSQIVLTQSPAIMSASPGEKVTMTCSASSSVSYMNWYQQKSGTSPKRWIYDTSKLASGVPAHFRGSGSGTSYSLTISGMEAEDAATYYCQQWSSNPFTFGSGTKLEINSSVVPVLQKVNSTTTKPVLRTPSPVHPTGTSQPQRPEDCRPRGSVKGTGLDFACDIYIWAPLAGICVALLLSLIITLICYHRSRKRVCKCPRPLVRQEGKPRPSEKIV

SEQ ID NO: 90 - protein, 304 aa, Artificial Sequence
  P3Z pro
MQIPQAPWPVVWAVLQLGWRPGWFLDSPDRPWNPPTFSPALLVVTEGDNATFTCSFSNTSESFVLNWYRMSPSNQTDKLAAFPEDRSQPGQDCRFRVTQLPNGRDFHMSVVRARRNDSGTYLCGAISLAPKAQIKESLRAELRVTERRAEVPTAHPSPSPRPAGQFQTLVVGVVGGLLGSLVLLVWVLAVIRVKFSRSADAPAYQQGQNQLYNELNLGRREEYDVLDKRRGRDPEMGGKPQRRKNPQEGLYNELQKDKMAEAYSEIGMKGERRRGKGHDGLYQGLSTATKDTYDALHMQALPPR